European Patent Application EP 4 289 436 A1, published December 13, 2023. Title: Pharmaceutical compound for prevention or treatment of liver fibrosis. Applicant: Medizinische Hochschule Hannover. The sequence listing filed with the application follows.

SEQUENCE LISTING (32 sequences)

SEQ ID NO: 1 - protein, 1130 aa, Homo sapiens
  hyaluronan synthetase (HAS2)
MAAAGQLCLLYLSAGLLSRLGAAFNLDTREDNVIRKYGDPGSLFGFSLAMHWQLQPEDKRLLLVGAPRAEALPLQRANRTGGLYSCDITARGPCTRIEFDNDADPTSESKEDQWMGVTVQSQGPGGKVVTCAHRYEKRQHVNTKQESRDIFGRCYVLSQNLRIEDDMDGGDWSFCDGRLRGHEKFGSCQQGVAATFTKDFHYIVFGAPGTYNWKGIVRVEQKNNTFFDMNIFEDGPYEVGGETEHDESLVPVPANSYLGLLFLTSVSYTDPDQFVYKTRPPREQPDTFPDVMMNSYLGFSLDSGKGIVSKDEITFVSGAPRANHSGAVVLLKRDMKSAHLLPEHIFDGEGLASSFGYDVAVVDLNKDGWQDIVIGAPQYFDRDGEVGGAVYVYMNQQGRWNNVKPIRLNGTKDSMFGIAVKNIGDINQDGYPDIAVGAPYDDLGKVFIYHGSANGINTKPTQVLKGISPYFGYSIAGNMDLDRNSYPDVAVGSLSDSVTIFRSRPVINIQKTITVTPNRIDLRQKTACGAPSGICLQVKSCFEYTANPAGYNPSISIVGTLEAEKERRKSGLSSRVQFRNQGSEPKYTQELTLKRQKQKVCMEETLWLQDNIRDKLRPIPITASVEIQEPSSRRRVNSLPEVLPILNSDEPKTAHIDVHFLKEGCGDDNVCNSNLKLEYKFCTREGNQDKFSYLPIQKGVPELVLKDQKDIALEITVTNSPSNPRNPTKDGDDAHEAKLIATFPDTLTYSAYRELRAFPEKQLSCVANQNGSQADCELGNPFKRNSNVTFYLVLSTTEVTFDTPDLDINLKLETTSNQDNLAPITAKAKVVIELLLSVSGVAKPSQVYFGGTVVGEQAMKSEDEVGSLIEYEFRVINLGKPLTNLGTATLNIQWPKEISNGKWLLYLVKVESKGLEKVTCEPQKEINSLNLTESHNSRKKREITEKQIDDNRKFSLFAERKYQTLNCSVNVNCVNIRCPLRGLDSKASLILRSRLWNSTFLEEYSKLNYLDILMRAFIDVTAAAENIRLPNAGTQVRVTVFPSKTVAQYSGVPWWIILVAILAGILMLALLVFILWKCGFFKRSRYDDSVPRYHAVRIRKEEREIKDEKYIDNLEKKQWITKWNENESYS

SEQ ID NO: 2 - protein, 552 aa, Homo sapiens
  integrin alpha-6 (ITGA6)
MHCERFLCILRIIGTTLFGVSLLLGITAAYIVGYQFIQTDNYYFSFGLYGAFLASHLIIQSLFAFLEHRKMKKSLETPIKLNKTVALCIAAYQEDPDYLRKCLQSVKRLTYPGIKVVMVIDGNSEDDLYMMDIFSEVMGRDKSATYIWKNNFHEKGPGETDESHKESSQHVTQLVLSNKSICIMQKWGGKREVMYTAFRALGRSVDYVQVCDSDTMLDPASSVEMVKVLEEDPMVGGVGGDVQILNKYDSWISFLSSVRYWMAFNIERACQSYFGCVQCISGPLGMYRNSLLHEFVEDWYNQEFMGNQCSFGDDRHLTNRVLSLGYATKYTARSKCLTETPIEYLRWLNQQTRWSKSYFREWLYNAMWFHKHHLWMTYEAIITGFFPFFLIATVIQLFYRGKIWNILLFLLTVQLVGLIKSSFASCLRGNIVMVFMSLYSVLYMSSLLPAKMFAIATINKAGWGTSGRKTIVVNFIGLIPVSVWFTILLGGVIFTIYKESKRPFSESKQTVLIVGTLLYACYWVMLLTLYVVLINKCGRRKKGQQYDMVLDV

SEQ ID NO: 3 - RNA, 22 nt, Homo sapiens
  mature miR-190b-5p
ugauauguuugauauuggguug

SEQ ID NO: 4 - RNA, 22 nt, Homo sapiens
  mature miR-296-3p
gaggguuggguggaggcucucc

SEQ ID NO: 5 - DNA, 1537 bp, Artificial Sequence
  AAV-Pdgfrb-miR-190b-5p
  promoter 1..1346: /note="Pdgfrb promoter"
  misc_feature 1385..1536: /note="Pre-miR-190b-5p"
  misc_feature 1441..1462: /note="mature miR-190b-5p"
acggtaccacagcttgagagggggactcagtcccatcatccttaagttcctggaatgatcttcctgtaagatttgctgtttctggaatctaagaatatactgtttttacacagggtctccctggatagccgagagccattttctgctgtgtctatctgggatggcaggcatccaccaccattctcagcttcttagtggtttttcagcttgcagtgagtatttagacagacacgcctttgatctgtactcatctgtgtgtggagatgaacaggagtcagacccaaagtttaaggtagcaagggagaaagctccaggcccaggtgaacggtcaggactcaacagtagcagtgtcagccctgggtctttctctagtgtgtcatcagccactcttttccttggggacctgcttagctaggaatgtctctccaactcaggtggcctcttactacagagtcccagcacacagtaccggtcctcaggtcctcaaacagggcagatgttcagtgaggtcactacacaaattatcagcacttcctttacagatggagaaattgaggcacagagaacgcgcgcgcgcgcgcgcacacacacacacacacacacacacacacacactagcaccccaggtaccatggtaaagggaggctccatttgacaggcatcaggcaagtggggcaggccactctaataaaagtgactcagtggctggcgtgggcagcggaatttctaaacatcctgaaagagccggtgaagggagggagcagagggaaaggaggaagaaaaacaagaaagttgggggaaaagaaagagaggaaaaaaaaaaaaaccctgaaattgaaaacagacacacgcgtccaccctccctgctccaccgctccccccacctccccgccttccccaagcttggccaatcagaatcggccctgcagcctttcccccaaagtgtgtggtggtggtggtggtggggcagagaaagcccacagtggtgtgagctctggggctgtctgtggccacagtcccggctaccctatctgggacctaggattgctctgggagtaactttgagagagaggagaacagagaggaaacagtccagagccagagcgggcccagaccagtcgtcagtctcctgcctgccagctagacctagggcggcccctcgggctgctccgctcctcccggaggatgcttttggagtgaggaggggccgggctgcttctcacccctgagcaccctctccattcccctgattctctcagggttttccgcaatcaggccagcccttctactgctgtccgttttttgggtccagcaaaataacagaagacagcgaggtggacttcctgctcactatagggcggccgggaattcgtcgactggatccctttgcaactggaaggaaggcagatgacccccaaagctctcctgcctgcttctgtgtgatatgtttgatattgggttgtttaattaggaaccaactaaatgtcaaacatattcttacagcagcaggtgattcagcaccaccctctttcataca

SEQ ID NO: 6 - DNA, 1539 bp, Artificial Sequence
  AAV-Pdgfrb-296-3p
  promoter 1..1346: /note="Pdgfrb promoter"
  misc_feature 1385..1538: /note="Pre-miR-296-3p"
  misc_feature 1453..1474: /note="mature miR-296-3p"
acggtaccacagcttgagagggggactcagtcccatcatccttaagttcctggaatgatcttcctgtaagatttgctgtttctggaatctaagaatatactgtttttacacagggtctccctggatagccgagagccattttctgctgtgtctatctgggatggcaggcatccaccaccattctcagcttcttagtggtttttcagcttgcagtgagtatttagacagacacgcctttgatctgtactcatctgtgtgtggagatgaacaggagtcagacccaaagtttaaggtagcaagggagaaagctccaggcccaggtgaacggtcaggactcaacagtagcagtgtcagccctgggtctttctctagtgtgtcatcagccactcttttccttggggacctgcttagctaggaatgtctctccaactcaggtggcctcttactacagagtcccagcacacagtaccggtcctcaggtcctcaaacagggcagatgttcagtgaggtcactacacaaattatcagcacttcctttacagatggagaaattgaggcacagagaacgcgcgcgcgcgcgcgcacacacacacacacacacacacacacacacactagcaccccaggtaccatggtaaagggaggctccatttgacaggcatcaggcaagtggggcaggccactctaataaaagtgactcagtggctggcgtgggcagcggaatttctaaacatcctgaaagagccggtgaagggagggagcagagggaaaggaggaagaaaaacaagaaagttgggggaaaagaaagagaggaaaaaaaaaaaaaccctgaaattgaaaacagacacacgcgtccaccctccctgctccaccgctccccccacctccccgccttccccaagcttggccaatcagaatcggccctgcagcctttcccccaaagtgtgtggtggtggtggtggtggggcagagaaagcccacagtggtgtgagctctggggctgtctgtggccacagtcccggctaccctatctgggacctaggattgctctgggagtaactttgagagagaggagaacagagaggaaacagtccagagccagagcgggcccagaccagtcgtcagtctcctgcctgccagctagacctagggcggcccctcgggctgctccgctcctcccggaggatgcttttggagtgaggaggggccgggctgcttctcacccctgagcaccctctccattcccctgattctctcagggttttccgcaatcaggccagcccttctactgctgtccgttttttgggtccagcaaaataacagaagacagcgaggtggacttcctgctcactatagggcggccgggaattcgtcgactggatcctcatgtgggaggtgaggagaaaggacccttccagagggccccccctcaatcctgttgtgcctaattcagagggttgggtggaggctctcctgaagggctctgaagagcgctgcacccgcagctgtgtgccaggagtggagacaggacagtcgata

SEQ ID NO: 7 - DNA, 814 bp, Artificial Sequence
  AAV-Cmv-296-3p
  enhancer 1..380: /note="CMV enhancer"
  promoter 381..584: /note="CMV promoter"
  misc_feature 656..809: /note="Pre-miR-296-3p"
  misc_feature 724..745: /note="mature miR-296-3p"
gacattgattattgactagttattaatagtaatcaattacggggtcattagttcatagcccatatatggagttccgcgttacataacttacggtaaatggcccgcctggctgaccgcccaacgacccccgcccattgacgtcaataatgacgtatgttcccatagtaacgccaatagggactttccattgacgtcaatgggtggagtatttacggtaaactgcccacttggcagtacatcaagtgtatcatatgccaagtccgccccctattgacgtcaatgacggtaaatggcccgcctggcattatgcccagtacatgaccttacgggactttcctacttggcagtacatctacgtattagtcatcgctattaccatggtgatgcggttttggcagtacaccaatgggcgtggatagcggtttgactcacggggatttccaagtctccaccccattgacgtcaatgggagtttgttttggcaccaaaatcaacgggactttccaaaatgtcgtaataaccccgccccgttgacgcaaatgggcggtaggcgtgtacggtgggaggtctatataagcagagctcgtttagtgaaccgtcagaattttgtaatacgactcactatagggcggccgggaattcgtcgactggatcctcatgtgggaggtgaggagaaaggacccttccagagggccccccctcaatcctgttgtgcctaattcagagggttgggtggaggctctcctgaagggctctgaagagcgctgcacccgcagctgtgtgccaggagtggagacaggacagtcgataagct

SEQ ID NO: 8 - DNA, 812 bp, Artificial Sequence
  AAV-Cmv-miR-190b-5p
  enhancer 1..380: /note="CMV enhancer"
  promoter 381..584: /note="CMV promoter"
  misc_feature 656..807: /note="pre-miR-190b-5p"
  misc_RNA 712..733: /note="mature miR-19b-5p"
gacattgattattgactagttattaatagtaatcaattacggggtcattagttcatagcccatatatggagttccgcgttacataacttacggtaaatggcccgcctggctgaccgcccaacgacccccgcccattgacgtcaataatgacgtatgttcccatagtaacgccaatagggactttccattgacgtcaatgggtggagtatttacggtaaactgcccacttggcagtacatcaagtgtatcatatgccaagtccgccccctattgacgtcaatgacggtaaatggcccgcctggcattatgcccagtacatgaccttacgggactttcctacttggcagtacatctacgtattagtcatcgctattaccatggtgatgcggttttggcagtacaccaatgggcgtggatagcggtttgactcacggggatttccaagtctccaccccattgacgtcaatgggagtttgttttggcaccaaaatcaacgggactttccaaaatgtcgtaataaccccgccccgttgacgcaaatgggcggtaggcgtgtacggtgggaggtctatataagcagagctcgtttagtgaaccgtcagaattttgtaatacgactcactatagggcggccgggaattcgtcgactggatccctttgcaactggaaggaaggcagatgacccccaaagctctcctgcctgcttctgtgtgatatgtttgatattgggttgtttaattaggaaccaactaaatgtcaaacatattcttacagcagcaggtgattcagcaccaccctctttcatacaagct

SEQ ID NO: 9 - DNA, 20 bp, Artificial Sequence
  Acta2 forward primer
gttcagtggtgcctctgtca

SEQ ID NO: 10 - DNA, 20 bp, Artificial Sequence
  Acta2 reverse primer
actgggacgacatggaaaag

SEQ ID NO: 11 - DNA, 18 bp, Artificial Sequence
  Actb forward primer
ctgtattcccctccatcg

SEQ ID NO: 12 - DNA, 20 bp, Artificial Sequence
  Actb reverse primer
agttggtaacaatgccatgt

SEQ ID NO: 13 - DNA, 20 bp, Artificial Sequence
  Col1a1 forward primer
taggccattgtgtatgcagc

SEQ ID NO: 14 - DNA, 21 bp, Artificial Sequence
  Col1a1 reverse primer
acatgttcagctttgtggacc

SEQ ID NO: 15 - DNA, 19 bp, Artificial Sequence
  Gapdh forward primer
tgcccccatgtttgtgatg

SEQ ID NO: 16 - DNA, 19 bp, Artificial Sequence
  Gapdh reverse primer
tgtggtcatgagcccttcc

SEQ ID NO: 17 - DNA, 20 bp, Artificial Sequence
  Has2 forward primer
gaaaggcaaccacagcgaag

SEQ ID NO: 18 - DNA, 21 bp, Artificial Sequence
  Has2 reverse primer
acatcaacctacaasgccggg

SEQ ID NO: 19 - DNA, 20 bp, Artificial Sequence
  Itga6 forward primer
caggttcgagtgacggtgtt

SEQ ID NO: 20 - DNA, 21 bp, Artificial Sequence
  Itga6 reverse primer
ctcagccttgtgataggtggc

SEQ ID NO: 21 - DNA, 18 bp, Artificial Sequence
  Rpl4 forward primer
cgctggtggttgaagata

SEQ ID NO: 22 - DNA, 18 bp, Artificial Sequence
  Rpl4 reverse primer
cggtttctcattttgccc

SEQ ID NO: 23 - DNA, 24 bp, Artificial Sequence
  S100a6 forward primer
tccgtgtttagttttcccttctgg

SEQ ID NO: 24 - DNA, 20 bp, Artificial Sequence
  S100a6 reverse primer
atgttcgtttgccttgcctc

SEQ ID NO: 25 - DNA, 20 bp, Artificial Sequence
  Tgfbr1 forward primer
gtggaaatcaacgggatcag

SEQ ID NO: 26 - DNA, 20 bp, Artificial Sequence
  Tgfbr1 reverse primer
acttccaacccaggtccttc

SEQ ID NO: 27 - DNA, 21 bp, Artificial Sequence
  HAS2 forward primer
tatcactgctgctgggacttg

SEQ ID NO: 28 - DNA, 20 bp, Artificial Sequence
  HAS2 reverse primer
gggcaaaacactttcaggcg

SEQ ID NO: 29 - DNA, 21 bp, Artificial Sequence
  ITGA6 forward primer
gagcttttgtgatgggcgatt

SEQ ID NO: 30 - DNA, 22 bp, Artificial Sequence
  ITGA6 reverse primer
ctctccaccaacttcataaggc

SEQ ID NO: 31 - DNA, 21 bp, Artificial Sequence
  GAPDH forward primer
tcttccaggagcgagatccct

SEQ ID NO: 32 - DNA, 22 bp, Artificial Sequence
  GAPDH reverse primer
tggtcatgagtccttccacgat